European Patent Specification EP 3 850 946 B1, published September 27, 2023. Title: NON-HUMAN ANIMALS HAVING A HUMANIZED CLUSTER OF DIFFERENTIATION 47 GENE. Applicant: REGENERON PHARMACEUTICALS, INC. The sequence listing filed with the application follows.

SEQUENCE LISTING (36 sequences)

SEQ ID NO: 1 - DNA, 5591 bp, Mus musculus
gcctacaccgggagagcagggaggaggagttggactgaggttgggcggctccgaggtccagggcgagcttggccagagggagtagagagcagcggggctgcgcagggacgcgtgccgtgagttccggtgagcgtgtgtgtcccatgctcccgtctttcaggccggcccaggacacgaagccggaagagagctggctggagggacgggggccgtgagcagagagtgcaacccgcgcagccccggggacaggctgattcttggcgctctccgccggagcctgcccagggctgggtgtgaggctggcgtcacgtcaacgagcagaggcggccaggcggggcggagtgcgcgtgcgcggggcggcgagcacgcgcgcgcgcgcacccccgggcagcctgggcggccgctcctgcctgtcactgctgcggcgctgctggtcggtcgtttcccttgaaggcagcagcggaggcggcggctgctccagacacctgcggcggcgaccccccggcggcgcggagatgtggcccttggcggcggcgctgttgctgggctcctgctgctgcggttcagctcaactactgtttagtaacgtcaactccatagagttcacttcatgcaatgaaactgtggtcatcccttgcatcgtccgtaatgtggaggcgcaaagcaccgaagaaatgtttgtgaagtggaagttgaacaaatcgtatattttcatctatgatggaaataaaaatagcactactacagatcaaaactttaccagtgcaaaaatctcagtctcagacttaatcaatggcattgcctctttgaaaatggataagcgcgatgccatggtgggaaactacacttgcgaagtgacagagttatccagagaaggcaaaacagttatagagctgaaaaaccgcacggccttcaacactgaccaaggatcagcctgttcttacgaggaggagaaaggaggttgcaaattagtttcgtggttttctccaaatgaaaagatcctcattgttattttcccaattttggctatactcctgttctggggaaagtttggtattttaacactcaaatataaatccagccatacgaataagagaatcattctgctgctcgttgccgggctggtgctcacagtcatcgtggttgttggagccatccttctcatcccaggagaaaagcccgtgaagaatgcttctggacttggcctcattgtaatctctacggggatattaatactacttcagtacaatgtgtttatgacagcttttggaatgacctctttcaccattgccatattgatcactcaagtgctgggctacgtccttgctttggtcgggctgtgtctctgcatcatggcatgtgagccagtgcacggcccccttttgatttcaggtttggggatcatagctctagcagaactacttggattagtttatatgaagtttgtcgaataggtgaagggaagtgacggactgtaacttggaagtcagaaatggaagaatacagttgtctaagcaccaggtcttcacgactcacagctggaaggaacagacaacagtaactgacttccatccaggaaaacatgtcacataaatgattactaagtttatattcaaagcagctgtactttacataataaaaaaaatatgatgtgctgtgtaaccaattggaatcccatttttctattgtttctactcaactaggggcaaacgtttcaggggcaacttccaagaatgatgcttgttagatcctagagtctctgaacactgagtttaaattgattccgagtgagactcgccaagcactaacctgagggttagttacccagagatacctatgaaaaacagtggtatccagcaagccttagtaaactcaggttgccagcagctttgccacttccgctgctagctgaataacaagactgccacttctgggtcatagtgatagagactgaagtagaaaaacgaatgtggttgggcaaatcccgtgtggcccctctgtgtgctatgatattgatggcactggtgtcttcattcttgggggttgccatcattcacacacacccctttgacatacagtgcaccccagttttgaatacattttttttgcaccctgtcccgttctgctactttgatttgcgttatgatatatatatatatatataataccttttctcctctttaaacatggtcctgtgacacaatagtcagttgcagaaaggagccagacttattcgcaaagcactgtgctcaaactcttcagaaaaaaaggaaaaaaaaaaaaagctatagttgtaacatatgtattccagacctctggtttaaaggcaaaagaaaaaaaatctacagtgtttcttctcatgttttctgatcggaggcatgacaaagcaagactgaaatctgaactgtgtctcctgcatggcaacacgtgtctccgtcaggccctcgcaaggcccggggagggggttctacgcctcttgtctctttgttgcatgctgaacactcatcgccttcctactgtatcctgcctcctgcagcctccctcttcctcctcctcttcctcttcctcctcttcctcctcctcctcctcttcctccaagtttgaaaggtcaaacaaaactaccacattccctacccagttagaagaaaaccaccgtcctgacagttgtgatcgcatggagtacttttagattattagcacctgtttttacctcgtttgtgggcgtgtttgtatgtgcacatgtatgaagtcggcacatgcaccttctgtatgggcagaggcgtggcatctacagaagagcagatgccaactttgtgcttttagtgaatacattaaaaaaaaaaaaccaacggtccttattgagtggaattctatttgatgcaaatatttgagctctttaagactttaaaactagataatgtgccaagcttttaggactgctcaccagtgccctctgaagaaacaccagtactttttcctgtttgtgtaataaaggcatatttgtatttgtgtttgcatcactaatggttatttcttcttagtccactgaatgtttccatgtgcctctcgtatgccaaactttttgtcatctttcatgtggggaccaaatggtttgtctgtggcaaacctaaacctatgacctgctgaggcctctcagaaaactgaccacagtaccaagatagtacttcgcaaagaaaagtaggttccctccctggttttgtagctgtcgccaatattagcgtaattccaaggagctgaacgcctttatataaatctgatggcacctgatgcttttagttctgaaaatatttacactcggatcatgttgttgatgacttaaacaaagttttgatgaagagagcaaaaaaaaagcaggtggatttggaacagtttcagggttttttttgttttttgttttttgtttttgtttttttttttttatttttgtttttctgttctctgttagaaaagtcaggtgttctctgtcaggctatctttatagtcaattttttttacgaactaaagtagtaccttttaatatgtagtcaacgcccctctgctcggggttcagttttgggtcttaaccagctgtcatgttctctatgctgcctgccacttgaggcactgagtgccctagacagtcccatcggtggtagccagggaaacgaaagacgaactcaactcttgctcctaataatcaactctctgtatgaaggatggcagcattaagagtcctcctgcctgggcattattgggccagttcaccctctttaaatcaaacccgcagtggctcccagttctcgtcccatcagatttaaattgctaacagtatggggggcaccacgcatctgttttgtcccacaatgcgcttttctctcccaaatcccgatttctgctgtcatagcctctattcaatttttatttattgtctgccctccacttatacaatcgtagagagcaatgccatttgtcactttctgcaacagttttttgagcctttatggctgaatcccatttttcttctctttcaaactgtttgctccattgctcctcccgcacggctgtccgtacagtcatcccatccatctgggggcctctttcatctctcacccttcctggtgcttcgtggatctctgcttacctctgtgggtttttttttttttttttgacttattcttctcactggactttaagattacttccacagcgaaagtgctgcctcccttttctgcccgcagtgttctgcgtactttagatactactcagtgctgacatttgatggcaaaagttgcctgcacttaaatttctctttttaatagggtgaactagagttggagtttttttctcttttttctcttttctctctctctctctctctctctctctctctctctctctctctccctccctccctccctccctccctccctccctctctctctctttttctttctttctttctttctttctttctttctttctttctttctttctttctttttttgacaaatctcacaggctttgagaattataaaaggtgacagttcacctgaaaatcacaggtctggtctgtttaaattgttgagaaatatccgattaaaagtcttgtggctgtgtcctaataggctctctttcaggacgttgtagtcaatagagtggctgaaccatacttgagtttataaagctcaaaaactgatgcacccactctgctattatcgtgttagtaagagttcagctgtatatcattgtctaggtttatcttgtcctacagtgggtattcaaatatggccaccagaggatatgtgtaaatataagcacctgtatttgcctgttgttgagaactggagggaaaacaaaaaatgtctggcaaccctttgcctttttaaccgtaattaattgacagtttatttagagataagagttttcaaaaatctcttaactgccacaacccacagagggtcttgttttgccatcttcagtggctcacagatatgatccaagttaacttgaaagagatgagcagtacccaggaaattgtcctgcctttaactctggctgtccttaattatgactgtttaatgctgaattttccatccgtctagtgtttgagggtaaagaaaagccttttttaaataagtatttctgtaaaacggcatcggtgggatcttctgtgttgctatcacgggtgaaagagggaaacatttcttatttttattaagcagagcattatttacagaaagccattgttgagaattagttcccacatcatataaatatccattaaccattctaaattgtaagagaactccagtgttgctatgcacaaggaactctcctgggggcctttttttgcatagcaattaaaggtatgctatttgtcagtagccattttttgcagtgatttaaagaccaaagttgttttacagctgtgttacccttaaaggttttttttttatgtattaaatcaatttatcactgtttgaagctttgaatacctgcaatctttgccaagatacttttttatttaaaaaaataactgtgtaaatattaccctgtaatattatatatacttaataaaacattttaagcta

SEQ ID NO: 2 - protein, 312 aa, Mus musculus
MWPLAAALLLGSCCCGSAQLLFSNVNSIEFTSCNETVVIPCIVRNVEAQSTEEMFVKWKLNKSYIFIYDGNKNSTTTDQNFTSAKISVSDLINGIASLKMDKRDAMVGNYTCEVTELSREGKTVIELKNRTAFNTDQGSACSYEEEKGGCKLVSWFSPNEKILIVIFPILAILLFWGKFGILTLKYKSSHTNKRIILLLVAGLVLTVIVVVGAILLIPGEKPVKNASGLGLIVISTGILILLQYNVFMTAFGMTSFTIAILITQVLGYVLALVGLCLCIMACEPVHGPLLISGLGIIALAELLGLVYMKFVE

SEQ ID NO: 3 - DNA, 5560 bp, Mus musculus
gcctacaccgggagagcagggaggaggagttggactgaggttgggcggctccgaggtccagggcgagcttggccagagggagtagagagcagcggggctgcgcagggacgcgtgccgtgagttccggtgagcgtgtgtgtcccatgctcccgtctttcaggccggcccaggacacgaagccggaagagagctggctggagggacgggggccgtgagcagagagtgcaacccgcgcagccccggggacaggctgattcttggcgctctccgccggagcctgcccagggctgggtgtgaggctggcgtcacgtcaacgagcagaggcggccaggcggggcggagtgcgcgtgcgcggggcggcgagcacgcgcgcgcgcgcacccccgggcagcctgggcggccgctcctgcctgtcactgctgcggcgctgctggtcggtcgtttcccttgaaggcagcagcggaggcggcggctgctccagacacctgcggcggcgaccccccggcggcgcggagatgtggcccttggcggcggcgctgttgctgggctcctgctgctgcggttcagctcaactactgtttagtaacgtcaactccatagagttcacttcatgcaatgaaactgtggtcatcccttgcatcgtccgtaatgtggaggcgcaaagcaccgaagaaatgtttgtgaagtggaagttgaacaaatcgtatattttcatctatgatggaaataaaaatagcactactacagatcaaaactttaccagtgcaaaaatctcagtctcagacttaatcaatggcattgcctctttgaaaatggataagcgcgatgccatggtgggaaactacacttgcgaagtgacagagttatccagagaaggcaaaacagttatagagctgaaaaaccgcacggtttcgtggttttctccaaatgaaaagatcctcattgttattttcccaattttggctatactcctgttctggggaaagtttggtattttaacactcaaatataaatccagccatacgaataagagaatcattctgctgctcgttgccgggctggtgctcacagtcatcgtggttgttggagccatccttctcatcccaggagaaaagcccgtgaagaatgcttctggacttggcctcattgtaatctctacggggatattaatactacttcagtacaatgtgtttatgacagcttttggaatgacctctttcaccattgccatattgatcactcaagtgctgggctacgtccttgctttggtcgggctgtgtctctgcatcatggcatgtgagccagtgcacggcccccttttgatttcaggtttggggatcatagctctagcagaactacttggattagtttatatgaagtttgtcgcttccaaccagaggactatccaacctcctaggaataggtgaagggaagtgacggactgtaacttggaagtcagaaatggaagaatacagttgtctaagcaccaggtcttcacgactcacagctggaaggaacagacaacagtaactgacttccatccaggaaaacatgtcacataaatgattactaagtttatattcaaagcagctgtactttacataataaaaaaaatatgatgtgctgtgtaaccaattggaatcccatttttctattgtttctactcaactaggggcaaacgtttcaggggcaacttccaagaatgatgcttgttagatcctagagtctctgaacactgagtttaaattgattccgagtgagactcgccaagcactaacctgagggttagttacccagagatacctatgaaaaacagtggtatccagcaagccttagtaaactcaggttgccagcagctttgccacttccgctgctagctgaataacaagactgccacttctgggtcatagtgatagagactgaagtagaaaaacgaatgtggttgggcaaatcccgtgtggcccctctgtgtgctatgatattgatggcactggtgtcttcattcttgggggttgccatcattcacacacacccctttgacatacagtgcaccccagttttgaatacattttttttgcaccctgtcccgttctgctactttgatttgcgttatgatatatatatatatatataataccttttctcctctttaaacatggtcctgtgacacaatagtcagttgcagaaaggagccagacttattcgcaaagcactgtgctcaaactcttcagaaaaaaaggaaaaaaaaaaaaagctatagttgtaacatatgtattccagacctctggtttaaaggcaaaagaaaaaaaatctacagtgtttcttctcatgttttctgatcggaggcatgacaaagcaagactgaaatctgaactgtgtctcctgcatggcaacacgtgtctccgtcaggccctcgcaaggcccggggagggggttctacgcctcttgtctctttgttgcatgctgaacactcatcgccttcctactgtatcctgcctcctgcagcctccctcttcctcctcctcttcctcttcctcctcttcctcctcctcctcctcttcctccaagtttgaaaggtcaaacaaaactaccacattccctacccagttagaagaaaaccaccgtcctgacagttgtgatcgcatggagtacttttagattattagcacctgtttttacctcgtttgtgggcgtgtttgtatgtgcacatgtatgaagtcggcacatgcaccttctgtatgggcagaggcgtggcatctacagaagagcagatgccaactttgtgcttttagtgaatacattaaaaaaaaaaaaccaacggtccttattgagtggaattctatttgatgcaaatatttgagctctttaagactttaaaactagataatgtgccaagcttttaggactgctcaccagtgccctctgaagaaacaccagtactttttcctgtttgtgtaataaaggcatatttgtatttgtgtttgcatcactaatggttatttcttcttagtccactgaatgtttccatgtgcctctcgtatgccaaactttttgtcatctttcatgtggggaccaaatggtttgtctgtggcaaacctaaacctatgacctgctgaggcctctcagaaaactgaccacagtaccaagatagtacttcgcaaagaaaagtaggttccctccctggttttgtagctgtcgccaatattagcgtaattccaaggagctgaacgcctttatataaatctgatggcacctgatgcttttagttctgaaaatatttacactcggatcatgttgttgatgacttaaacaaagttttgatgaagagagcaaaaaaaaagcaggtggatttggaacagtttcagggttttttttgttttttgttttttgtttttgtttttttttttttatttttgtttttctgttctctgttagaaaagtcaggtgttctctgtcaggctatctttatagtcaattttttttacgaactaaagtagtaccttttaatatgtagtcaacgcccctctgctcggggttcagttttgggtcttaaccagctgtcatgttctctatgctgcctgccacttgaggcactgagtgccctagacagtcccatcggtggtagccagggaaacgaaagacgaactcaactcttgctcctaataatcaactctctgtatgaaggatggcagcattaagagtcctcctgcctgggcattattgggccagttcaccctctttaaatcaaacccgcagtggctcccagttctcgtcccatcagatttaaattgctaacagtatggggggcaccacgcatctgttttgtcccacaatgcgcttttctctcccaaatcccgatttctgctgtcatagcctctattcaatttttatttattgtctgccctccacttatacaatcgtagagagcaatgccatttgtcactttctgcaacagttttttgagcctttatggctgaatcccatttttcttctctttcaaactgtttgctccattgctcctcccgcacggctgtccgtacagtcatcccatccatctgggggcctctttcatctctcacccttcctggtgcttcgtggatctctgcttacctctgtgggtttttttttttttttttgacttattcttctcactggactttaagattacttccacagcgaaagtgctgcctcccttttctgcccgcagtgttctgcgtactttagatactactcagtgctgacatttgatggcaaaagttgcctgcacttaaatttctctttttaatagggtgaactagagttggagtttttttctcttttttctcttttctctctctctctctctctctctctctctctctctctctctctccctccctccctccctccctccctccctccctctctctctctttttctttctttctttctttctttctttctttctttctttctttctttctttctttttttgacaaatctcacaggctttgagaattataaaaggtgacagttcacctgaaaatcacaggtctggtctgtttaaattgttgagaaatatccgattaaaagtcttgtggctgtgtcctaataggctctctttcaggacgttgtagtcaatagagtggctgaaccatacttgagtttataaagctcaaaaactgatgcacccactctgctattatcgtgttagtaagagttcagctgtatatcattgtctaggtttatcttgtcctacagtgggtattcaaatatggccaccagaggatatgtgtaaatataagcacctgtatttgcctgttgttgagaactggagggaaaacaaaaaatgtctggcaaccctttgcctttttaaccgtaattaattgacagtttatttagagataagagttttcaaaaatctcttaactgccacaacccacagagggtcttgttttgccatcttcagtggctcacagatatgatccaagttaacttgaaagagatgagcagtacccaggaaattgtcctgcctttaactctggctgtccttaattatgactgtttaatgctgaattttccatccgtctagtgtttgagggtaaagaaaagccttttttaaataagtatttctgtaaaacggcatcggtgggatcttctgtgttgctatcacgggtgaaagagggaaacatttcttatttttattaagcagagcattatttacagaaagccattgttgagaattagttcccacatcatataaatatccattaaccattctaaattgtaagagaactccagtgttgctatgcacaaggaactctcctgggggcctttttttgcatagcaattaaaggtatgctatttgtcagtagccattttttgcagtgatttaaagaccaaagttgttttacagctgtgttacccttaaaggttttttttttatgtattaaatcaatttatcactgtttgaagctttgaatacctgcaatctttgccaagatacttttttatttaaaaaaataactgtgtaaatattaccctgtaatattatatatacttaataaaacattttaagcta

SEQ ID NO: 4 - protein, 303 aa, Mus musculus
MWPLAAALLLGSCCCGSAQLLFSNVNSIEFTSCNETVVIPCIVRNVEAQSTEEMFVKWKLNKSYIFIYDGNKNSTTTDQNFTSAKISVSDLINGIASLKMDKRDAMVGNYTCEVTELSREGKTVIELKNRTVSWFSPNEKILIVIFPILAILLFWGKFGILTLKYKSSHTNKRIILLLVAGLVLTVIVVVGAILLIPGEKPVKNASGLGLIVISTGILILLQYNVFMTAFGMTSFTIAILITQVLGYVLALVGLCLCIMACEPVHGPLLISGLGIIALAELLGLVYMKFVASNQRTIQPPRNR

SEQ ID NO: 5 - DNA, 5648 bp, Mus musculus
gcctacaccgggagagcagggaggaggagttggactgaggttgggcggctccgaggtccagggcgagcttggccagagggagtagagagcagcggggctgcgcagggacgcgtgccgtgagttccggtgagcgtgtgtgtcccatgctcccgtctttcaggccggcccaggacacgaagccggaagagagctggctggagggacgggggccgtgagcagagagtgcaacccgcgcagccccggggacaggctgattcttggcgctctccgccggagcctgcccagggctgggtgtgaggctggcgtcacgtcaacgagcagaggcggccaggcggggcggagtgcgcgtgcgcggggcggcgagcacgcgcgcgcgcgcacccccgggcagcctgggcggccgctcctgcctgtcactgctgcggcgctgctggtcggtcgtttcccttgaaggcagcagcggaggcggcggctgctccagacacctgcggcggcgaccccccggcggcgcggagatgtggcccttggcggcggcgctgttgctgggctcctgctgctgcggttcagctcaactactgtttagtaacgtcaactccatagagttcacttcatgcaatgaaactgtggtcatcccttgcatcgtccgtaatgtggaggcgcaaagcaccgaagaaatgtttgtgaagtggaagttgaacaaatcgtatattttcatctatgatggaaataaaaatagcactactacagatcaaaactttaccagtgcaaaaatctcagtctcagacttaatcaatggcattgcctctttgaaaatggataagcgcgatgccatggtgggaaactacacttgcgaagtgacagagttatccagagaaggcaaaacagttatagagctgaaaaaccgcacggccttcaacactgaccaaggatcagcctgttcttacgaggaggagaaaggaggttgcaaattagtttcgtggttttctccaaatgaaaagatcctcattgttattttcccaattttggctatactcctgttctggggaaagtttggtattttaacactcaaatataaatccagccatacgaataagagaatcattctgctgctcgttgccgggctggtgctcacagtcatcgtggttgttggagccatccttctcatcccaggagaaaagcccgtgaagaatgcttctggacttggcctcattgtaatctctacggggatattaatactacttcagtacaatgtgtttatgacagcttttggaatgacctctttcaccattgccatattgatcactcaagtgctgggctacgtccttgctttggtcgggctgtgtctctgcatcatggcatgtgagccagtgcacggcccccttttgatttcaggtttggggatcatagctctagcagaactacttggattagtttatatgaagtttgtcgcttccaaccagaggactatccaacctcctaggaaagctgtagaggaaccccttaacgaataggtgaagggaagtgacggactgtaacttggaagtcagaaatggaagaatacagttgtctaagcaccaggtcttcacgactcacagctggaaggaacagacaacagtaactgacttccatccaggaaaacatgtcacataaatgattactaagtttatattcaaagcagctgtactttacataataaaaaaaatatgatgtgctgtgtaaccaattggaatcccatttttctattgtttctactcaactaggggcaaacgtttcaggggcaacttccaagaatgatgcttgttagatcctagagtctctgaacactgagtttaaattgattccgagtgagactcgccaagcactaacctgagggttagttacccagagatacctatgaaaaacagtggtatccagcaagccttagtaaactcaggttgccagcagctttgccacttccgctgctagctgaataacaagactgccacttctgggtcatagtgatagagactgaagtagaaaaacgaatgtggttgggcaaatcccgtgtggcccctctgtgtgctatgatattgatggcactggtgtcttcattcttgggggttgccatcattcacacacacccctttgacatacagtgcaccccagttttgaatacattttttttgcaccctgtcccgttctgctactttgatttgcgttatgatatatatatatatatataataccttttctcctctttaaacatggtcctgtgacacaatagtcagttgcagaaaggagccagacttattcgcaaagcactgtgctcaaactcttcagaaaaaaaggaaaaaaaaaaaaagctatagttgtaacatatgtattccagacctctggtttaaaggcaaaagaaaaaaaatctacagtgtttcttctcatgttttctgatcggaggcatgacaaagcaagactgaaatctgaactgtgtctcctgcatggcaacacgtgtctccgtcaggccctcgcaaggcccggggagggggttctacgcctcttgtctctttgttgcatgctgaacactcatcgccttcctactgtatcctgcctcctgcagcctccctcttcctcctcctcttcctcttcctcctcttcctcctcctcctcctcttcctccaagtttgaaaggtcaaacaaaactaccacattccctacccagttagaagaaaaccaccgtcctgacagttgtgatcgcatggagtacttttagattattagcacctgtttttacctcgtttgtgggcgtgtttgtatgtgcacatgtatgaagtcggcacatgcaccttctgtatgggcagaggcgtggcatctacagaagagcagatgccaactttgtgcttttagtgaatacattaaaaaaaaaaaaccaacggtccttattgagtggaattctatttgatgcaaatatttgagctctttaagactttaaaactagataatgtgccaagcttttaggactgctcaccagtgccctctgaagaaacaccagtactttttcctgtttgtgtaataaaggcatatttgtatttgtgtttgcatcactaatggttatttcttcttagtccactgaatgtttccatgtgcctctcgtatgccaaactttttgtcatctttcatgtggggaccaaatggtttgtctgtggcaaacctaaacctatgacctgctgaggcctctcagaaaactgaccacagtaccaagatagtacttcgcaaagaaaagtaggttccctccctggttttgtagctgtcgccaatattagcgtaattccaaggagctgaacgcctttatataaatctgatggcacctgatgcttttagttctgaaaatatttacactcggatcatgttgttgatgacttaaacaaagttttgatgaagagagcaaaaaaaaagcaggtggatttggaacagtttcagggttttttttgttttttgttttttgtttttgtttttttttttttatttttgtttttctgttctctgttagaaaagtcaggtgttctctgtcaggctatctttatagtcaattttttttacgaactaaagtagtaccttttaatatgtagtcaacgcccctctgctcggggttcagttttgggtcttaaccagctgtcatgttctctatgctgcctgccacttgaggcactgagtgccctagacagtcccatcggtggtagccagggaaacgaaagacgaactcaactcttgctcctaataatcaactctctgtatgaaggatggcagcattaagagtcctcctgcctgggcattattgggccagttcaccctctttaaatcaaacccgcagtggctcccagttctcgtcccatcagatttaaattgctaacagtatggggggcaccacgcatctgttttgtcccacaatgcgcttttctctcccaaatcccgatttctgctgtcatagcctctattcaatttttatttattgtctgccctccacttatacaatcgtagagagcaatgccatttgtcactttctgcaacagttttttgagcctttatggctgaatcccatttttcttctctttcaaactgtttgctccattgctcctcccgcacggctgtccgtacagtcatcccatccatctgggggcctctttcatctctcacccttcctggtgcttcgtggatctctgcttacctctgtgggtttttttttttttttttgacttattcttctcactggactttaagattacttccacagcgaaagtgctgcctcccttttctgcccgcagtgttctgcgtactttagatactactcagtgctgacatttgatggcaaaagttgcctgcacttaaatttctctttttaatagggtgaactagagttggagtttttttctcttttttctcttttctctctctctctctctctctctctctctctctctctctctctccctccctccctccctccctccctccctccctctctctctctttttctttctttctttctttctttctttctttctttctttctttctttctttctttttttgacaaatctcacaggctttgagaattataaaaggtgacagttcacctgaaaatcacaggtctggtctgtttaaattgttgagaaatatccgattaaaagtcttgtggctgtgtcctaataggctctctttcaggacgttgtagtcaatagagtggctgaaccatacttgagtttataaagctcaaaaactgatgcacccactctgctattatcgtgttagtaagagttcagctgtatatcattgtctaggtttatcttgtcctacagtgggtattcaaatatggccaccagaggatatgtgtaaatataagcacctgtatttgcctgttgttgagaactggagggaaaacaaaaaatgtctggcaaccctttgcctttttaaccgtaattaattgacagtttatttagagataagagttttcaaaaatctcttaactgccacaacccacagagggtcttgttttgccatcttcagtggctcacagatatgatccaagttaacttgaaagagatgagcagtacccaggaaattgtcctgcctttaactctggctgtccttaattatgactgtttaatgctgaattttccatccgtctagtgtttgagggtaaagaaaagccttttttaaataagtatttctgtaaaacggcatcggtgggatcttctgtgttgctatcacgggtgaaagagggaaacatttcttatttttattaagcagagcattatttacagaaagccattgttgagaattagttcccacatcatataaatatccattaaccattctaaattgtaagagaactccagtgttgctatgcacaaggaactctcctgggggcctttttttgcatagcaattaaaggtatgctatttgtcagtagccattttttgcagtgatttaaagaccaaagttgttttacagctgtgttacccttaaaggttttttttttatgtattaaatcaatttatcactgtttgaagctttgaatacctgcaatctttgccaagatacttttttatttaaaaaaataactgtgtaaatattaccctgtaatattatatatacttaataaaacattttaagcta

SEQ ID NO: 6 - protein, 331 aa, Mus musculus
MWPLAAALLLGSCCCGSAQLLFSNVNSIEFTSCNETVVIPCIVRNVEAQSTEEMFVKWKLNKSYIFIYDGNKNSTTTDQNFTSAKISVSDLINGIASLKMDKRDAMVGNYTCEVTELSREGKTVIELKNRTAFNTDQGSACSYEEEKGGCKLVSWFSPNEKILIVIFPILAILLFWGKFGILTLKYKSSHTNKRIILLLVAGLVLTVIVVVGAILLIPGEKPVKNASGLGLIVISTGILILLQYNVFMTAFGMTSFTIAILITQVLGYVLALVGLCLCIMACEPVHGPLLISGLGIIALAELLGLVYMKFVASNQRTIQPPRKAVEEPLNE

SEQ ID NO: 7 - DNA, 5618 bp, Mus musculus
gcctacaccgggagagcagggaggaggagttggactgaggttgggcggctccgaggtccagggcgagcttggccagagggagtagagagcagcggggctgcgcagggacgcgtgccgtgagttccggtgagcgtgtgtgtcccatgctcccgtctttcaggccggcccaggacacgaagccggaagagagctggctggagggacgggggccgtgagcagagagtgcaacccgcgcagccccggggacaggctgattcttggcgctctccgccggagcctgcccagggctgggtgtgaggctggcgtcacgtcaacgagcagaggcggccaggcggggcggagtgcgcgtgcgcggggcggcgagcacgcgcgcgcgcgcacccccgggcagcctgggcggccgctcctgcctgtcactgctgcggcgctgctggtcggtcgtttcccttgaaggcagcagcggaggcggcggctgctccagacacctgcggcggcgaccccccggcggcgcggagatgtggcccttggcggcggcgctgttgctgggctcctgctgctgcggttcagctcaactactgtttagtaacgtcaactccatagagttcacttcatgcaatgaaactgtggtcatcccttgcatcgtccgtaatgtggaggcgcaaagcaccgaagaaatgtttgtgaagtggaagttgaacaaatcgtatattttcatctatgatggaaataaaaatagcactactacagatcaaaactttaccagtgcaaaaatctcagtctcagacttaatcaatggcattgcctctttgaaaatggataagcgcgatgccatggtgggaaactacacttgcgaagtgacagagttatccagagaaggcaaaacagttatagagctgaaaaaccgcacggtttcgtggttttctccaaatgaaaagatcctcattgttattttcccaattttggctatactcctgttctggggaaagtttggtattttaacactcaaatataaatccagccatacgaataagagaatcattctgctgctcgttgccgggctggtgctcacagtcatcgtggttgttggagccatccttctcatcccaggagaaaagcccgtgaagaatgcttctggacttggcctcattgtaatctctacggggatattaatactacttcagtacaatgtgtttatgacagcttttggaatgacctctttcaccattgccatattgatcactcaagtgctgggctacgtccttgctttggtcgggctgtgtctctgcatcatggcatgtgagccagtgcacggcccccttttgatttcaggtttggggatcatagctctagcagaactacttggattagtttatatgaagtttgtcgcttccaaccagaggactatccaacctcctaggaaagctgtagaggaaccccttaacgcatttaaagagtcaaaaggaatgatgaatgacgaataggtgaagggaagtgacggactgtaacttggaagtcagaaatggaagaatacagttgtctaagcaccaggtcttcacgactcacagctggaaggaacagacaacagtaactgacttccatccaggaaaacatgtcacataaatgattactaagtttatattcaaagcagctgtactttacataataaaaaaaatatgatgtgctgtgtaaccaattggaatcccatttttctattgtttctactcaactaggggcaaacgtttcaggggcaacttccaagaatgatgcttgttagatcctagagtctctgaacactgagtttaaattgattccgagtgagactcgccaagcactaacctgagggttagttacccagagatacctatgaaaaacagtggtatccagcaagccttagtaaactcaggttgccagcagctttgccacttccgctgctagctgaataacaagactgccacttctgggtcatagtgatagagactgaagtagaaaaacgaatgtggttgggcaaatcccgtgtggcccctctgtgtgctatgatattgatggcactggtgtcttcattcttgggggttgccatcattcacacacacccctttgacatacagtgcaccccagttttgaatacattttttttgcaccctgtcccgttctgctactttgatttgcgttatgatatatatatatatatataataccttttctcctctttaaacatggtcctgtgacacaatagtcagttgcagaaaggagccagacttattcgcaaagcactgtgctcaaactcttcagaaaaaaaggaaaaaaaaaaaaagctatagttgtaacatatgtattccagacctctggtttaaaggcaaaagaaaaaaaatctacagtgtttcttctcatgttttctgatcggaggcatgacaaagcaagactgaaatctgaactgtgtctcctgcatggcaacacgtgtctccgtcaggccctcgcaaggcccggggagggggttctacgcctcttgtctctttgttgcatgctgaacactcatcgccttcctactgtatcctgcctcctgcagcctccctcttcctcctcctcttcctcttcctcctcttcctcctcctcctcctcttcctccaagtttgaaaggtcaaacaaaactaccacattccctacccagttagaagaaaaccaccgtcctgacagttgtgatcgcatggagtacttttagattattagcacctgtttttacctcgtttgtgggcgtgtttgtatgtgcacatgtatgaagtcggcacatgcaccttctgtatgggcagaggcgtggcatctacagaagagcagatgccaactttgtgcttttagtgaatacattaaaaaaaaaaaaccaacggtccttattgagtggaattctatttgatgcaaatatttgagctctttaagactttaaaactagataatgtgccaagcttttaggactgctcaccagtgccctctgaagaaacaccagtactttttcctgtttgtgtaataaaggcatatttgtatttgtgtttgcatcactaatggttatttcttcttagtccactgaatgtttccatgtgcctctcgtatgccaaactttttgtcatctttcatgtggggaccaaatggtttgtctgtggcaaacctaaacctatgacctgctgaggcctctcagaaaactgaccacagtaccaagatagtacttcgcaaagaaaagtaggttccctccctggttttgtagctgtcgccaatattagcgtaattccaaggagctgaacgcctttatataaatctgatggcacctgatgcttttagttctgaaaatatttacactcggatcatgttgttgatgacttaaacaaagttttgatgaagagagcaaaaaaaaagcaggtggatttggaacagtttcagggttttttttgttttttgttttttgtttttgtttttttttttttatttttgtttttctgttctctgttagaaaagtcaggtgttctctgtcaggctatctttatagtcaattttttttacgaactaaagtagtaccttttaatatgtagtcaacgcccctctgctcggggttcagttttgggtcttaaccagctgtcatgttctctatgctgcctgccacttgaggcactgagtgccctagacagtcccatcggtggtagccagggaaacgaaagacgaactcaactcttgctcctaataatcaactctctgtatgaaggatggcagcattaagagtcctcctgcctgggcattattgggccagttcaccctctttaaatcaaacccgcagtggctcccagttctcgtcccatcagatttaaattgctaacagtatggggggcaccacgcatctgttttgtcccacaatgcgcttttctctcccaaatcccgatttctgctgtcatagcctctattcaatttttatttattgtctgccctccacttatacaatcgtagagagcaatgccatttgtcactttctgcaacagttttttgagcctttatggctgaatcccatttttcttctctttcaaactgtttgctccattgctcctcccgcacggctgtccgtacagtcatcccatccatctgggggcctctttcatctctcacccttcctggtgcttcgtggatctctgcttacctctgtgggtttttttttttttttttgacttattcttctcactggactttaagattacttccacagcgaaagtgctgcctcccttttctgcccgcagtgttctgcgtactttagatactactcagtgctgacatttgatggcaaaagttgcctgcacttaaatttctctttttaatagggtgaactagagttggagtttttttctcttttttctcttttctctctctctctctctctctctctctctctctctctctctctccctccctccctccctccctccctccctccctctctctctctttttctttctttctttctttctttctttctttctttctttctttctttctttctttttttgacaaatctcacaggctttgagaattataaaaggtgacagttcacctgaaaatcacaggtctggtctgtttaaattgttgagaaatatccgattaaaagtcttgtggctgtgtcctaataggctctctttcaggacgttgtagtcaatagagtggctgaaccatacttgagtttataaagctcaaaaactgatgcacccactctgctattatcgtgttagtaagagttcagctgtatatcattgtctaggtttatcttgtcctacagtgggtattcaaatatggccaccagaggatatgtgtaaatataagcacctgtatttgcctgttgttgagaactggagggaaaacaaaaaatgtctggcaaccctttgcctttttaaccgtaattaattgacagtttatttagagataagagttttcaaaaatctcttaactgccacaacccacagagggtcttgttttgccatcttcagtggctcacagatatgatccaagttaacttgaaagagatgagcagtacccaggaaattgtcctgcctttaactctggctgtccttaattatgactgtttaatgctgaattttccatccgtctagtgtttgagggtaaagaaaagccttttttaaataagtatttctgtaaaacggcatcggtgggatcttctgtgttgctatcacgggtgaaagagggaaacatttcttatttttattaagcagagcattatttacagaaagccattgttgagaattagttcccacatcatataaatatccattaaccattctaaattgtaagagaactccagtgttgctatgcacaaggaactctcctgggggcctttttttgcatagcaattaaaggtatgctatttgtcagtagccattttttgcagtgatttaaagaccaaagttgttttacagctgtgttacccttaaaggttttttttttatgtattaaatcaatttatcactgtttgaagctttgaatacctgcaatctttgccaagatacttttttatttaaaaaaataactgtgtaaatattaccctgtaatattatatatacttaataaaacattttaagcta

SEQ ID NO: 8 - protein, 321 aa, Mus musculus
MWPLAAALLLGSCCCGSAQLLFSNVNSIEFTSCNETVVIPCIVRNVEAQSTEEMFVKWKLNKSYIFIYDGNKNSTTTDQNFTSAKISVSDLINGIASLKMDKRDAMVGNYTCEVTELSREGKTVIELKNRTVSWFSPNEKILIVIFPILAILLFWGKFGILTLKYKSSHTNKRIILLLVAGLVLTVIVVVGAILLIPGEKPVKNASGLGLIVISTGILILLQYNVFMTAFGMTSFTIAILITQVLGYVLALVGLCLCIMACEPVHGPLLISGLGIIALAELLGLVYMKFVASNQRTIQPPRKAVEEPLNAFKESKGMMNDE

SEQ ID NO: 9 - DNA, 5021 bp, Homo sapiens
agtgggagcgcgcgtgcgcgcggccgtgcagcctgggcagtgggtcctgcctgtgacgcgcggcggcggtcggtcctgcctgtaacggcggcggcggctgctgctccggacacctgcggcggcggcggcgaccccgcggcgggcgcggagatgtggcccctggtagcggcgctgttgctgggctcggcgtgctgcggatcagctcagctactatttaataaaacaaaatctgtagaattcacgttttgtaatgacactgtcgtcattccatgctttgttactaatatggaggcacaaaacactactgaagtatacgtaaagtggaaatttaaaggaagagatatttacacctttgatggagctctaaacaagtccactgtccccactgactttagtagtgcaaaaattgaagtctcacaattactaaaaggagatgcctctttgaagatggataagagtgatgctgtctcacacacaggaaactacacttgtgaagtaacagaattaaccagagaaggtgaaacgatcatcgagctaaaatatcgtgttgtttcatggttttctccaaatgaaaatattcttattgttattttcccaatttttgctatactcctgttctggggacagtttggtattaaaacacttaaatatagatccggtggtatggatgagaaaacaattgctttacttgttgctggactagtgatcactgtcattgtcattgttggagccattcttttcgtcccaggtgaatattcattaaagaatgctactggccttggtttaattgtgacttctacagggatattaatattacttcactactatgtgtttagtacagcgattggattaacctccttcgtcattgccatattggttattcaggtgatagcctatatcctcgctgtggttggactgagtctctgtattgcggcgtgtataccaatgcatggccctcttctgatttcaggtttgagtatcttagctctagcacaattacttggactagtttatatgaaatttgtggaataactgaagtgaagtgatggactccgatttggagagtagtaagacgtgaaaggaatacacttgtgtttaagcaccatggccttgatgattcactgttggggagaagaaacaagaaaagtaactggttgtcacctatgagacccttacgtgattgttagttaagtttttattcaaagcagctgtaatttagttaataaaataattatgatctatgttgtttgcccaattgagatccagttttttgttgttatttttaatcaattaggggcaatagtagaatggacaatttccaagaatgatgcctttcaggtcctagggcctctggcctctaggtaaccagtttaaattggttcagggtgataactacttagcactgccctggtgattacccagagatatctatgaaaaccagtggcttccatcaaacctttgccaactcaggttcacagcagctttgggcagttatggcagtatggcattagctgagaggtgtctgccacttctgggtcaatggaataataaattaagtacaggcaggaatttggttgggagcatcttgtatgatctccgtatgatgtgatattgatggagatagtggtcctcattcttgggggttgccattcccacattcccccttcaacaaacagtgtaacaggtccttcccagatttagggtacttttattgatggatatgttttccttttattcacataaccccttgaaaccctgtcttgtcctcctgttacttgcttctgctgtacaagatgtagcaccttttctcctctttgaacatggtctagtgacacggtagcaccagttgcaggaaggagccagacttgttctcagagcactgtgttcacacttttcagcaaaaatagctatggttgtaacatatgtattcccttcctctgatttgaaggcaaaaatctacagtgtttcttcacttcttttctgatctggggcatgaaaaaagcaagattgaaatttgaactatgagtctcctgcatggcaacaaaatgtgtgtcaccatcaggccaacaggccagcccttgaatggggatttattactgttgtatctatgttgcatgataaacattcatcaccttcctcctgtagtcctgcctcgtactccccttcccctatgattgaaaagtaaacaaaacccacatttcctatcctggttagaagaaaattaatgttctgacagttgtgatcgcctggagtacttttagacttttagcattcgttttttacctgtttgtggatgtgtgtttgtatgtgcatacgtatgagataggcacatgcatcttctgtatggacaaaggtggggtacctacaggagagcaaaggttaattttgtgcttttagtaaaaacatttaaatacaaagttctttattgggtggaattatatttgatgcaaatatttgatcacttaaaacttttaaaacttctaggtaatttgccacgctttttgactgctcaccaataccctgtaaaaatacgtaattcttcctgtttgtgtaataagatattcatatttgtagttgcattaataatagttatttcttagtccatcagatgttcccgtgtgcctcttttatgccaaattgattgtcatatttcatgttgggaccaagtagtttgcccatggcaaacctaaatttatgacctgctgaggcctctcagaaaactgagcatactagcaagacagctcttcttgaaaaaaaaaatatgtatacacaaatatatacgtatatctatatatacgtatgtatatacacacatgtatattcttccttgattgtgtagctgtccaaaataataacatatatagagggagctgtattcctttatacaaatctgatggctcctgcagcactttttccttctgaaaatatttacattttgctaacctagtttgttactttaaaaatcagttttgatgaaaggagggaaaagcagatggacttgaaaaagatccaagctcctattagaaaaggtatgaaaatctttatagtaaaattttttataaactaaagttgtaccttttaatatgtagtaaactctcatttatttggggttcgctcttggatctcatccatccattgtgttctctttaatgctgcctgccttttgaggcattcactgccctagacaatgccaccagagatagtgggggaaatgccagatgaaaccaactcttgctctcactagttgtcagcttctctggataagtgaccacagaagcaggagtcctcctgcttgggcatcattgggccagttccttctctttaaatcagatttgtaatggctcccaaattccatcacatcacatttaaattgcagacagtgttttgcacatcatgtatctgttttgtcccataatatgctttttactccctgatcccagtttctgctgttgactcttccattcagttttatttattgtgtgttctcacagtgacaccatttgtccttttctgcaacaacctttccagctacttttgccaaattctatttgtcttctccttcaaaacattctcctttgcagttcctcttcatctgtgtagctgctcttttgtctcttaacttaccattcctatagtactttatgcatctctgcttagttctattagttttttggccttgctcttctccttgattttaaaattccttctatagctagagcttttctttctttcattctctcttcctgcagtgttttgcatacatcagaagctaggtacataagttaaatgattgagagttggctgtatttagatttatcactttttaatagggtgagcttgagagttttctttctttctgttttttttttttgttttttttttttttttttttttttttttttttgactaatttcacatgctctaaaaaccttcaaaggtgattatttttctcctggaaactccaggtccattctgtttaaatccctaagaatgtcagaattaaaataacagggctatcccgtaattggaaatatttcttttttcaggatgctatagtcaatttagtaagtgaccaccaaattgttatttgcactaacaaagctcaaaacacgataagtttactcctccatctcagtaataaaaattaagctgtaatcaaccttctaggtttctcttgtcttaaaatgggtattcaaaaatggggatctgtggtgtatgtatggaaacacatactccttaatttacctgttgttggaaactggagaaatgattgtcgggcaaccgtttattttttattgtattttatttggttgagggatttttttataaacagttttacttgtgtcatattttaaaattactaactgccatcacctgctggggtcctttgttaggtcattttcagtgactaatagggataatccaggtaactttgaagagatgagcagtgagtgaccaggcagtttttctgcctttagctttgacagttcttaattaagatcattgaagaccagctttctcataaatttctctttttgaaaaaaagaaagcatttgtactaagctcctctgtaagacaacatcttaaatcttaaaagtgttgttatcatgactggtgagagaagaaaacattttgtttttattaaatggagcattatttacaaaaagccattgttgagaattagatcccacatcgtataaatatctattaaccattctaaataaagagaactccagtgttgctatgtgcaagatcctctcttggagcttttttgcatagcaattaaaggtgtgctatttgtcagtagccatttttttgcagtgatttgaagaccaaagttgttttacagctgtgttaccgttaaaggtttttttttttatatgtattaaatcaatttatcactgtttaaagctttgaatatctgcaatctttgccaaggtacttttttatttaaaaaaaaacataactttgtaaatattaccctgtaatattatatatacttaataaaacattttaagcta

SEQ ID NO: 10 - protein, 293 aa, Homo sapiens
MWPLVAALLLGSACCGSAQLLFNKTKSVEFTFCNDTVVIPCFVTNMEAQNTTEVYVKWKFKGRDIYTFDGALNKSTVPTDFSSAKIEVSQLLKGDASLKMDKSDAVSHTGNYTCEVTELTREGETIIELKYRVVSWFSPNENILIVIFPIFAILLFWGQFGIKTLKYRSGGMDEKTIALLVAGLVITVIVIVGAILFVPGEYSLKNATGLGLIVTSTGILILLHYYVFSTAIGLTSFVIAILVIQVIAYILAVVGLSLCIAACIPMHGPLLISGLSILALAQLLGLVYMKFVE

SEQ ID NO: 11 - DNA, 5288 bp, Homo sapiens
ggggagcaggcgggggagcgggcgggaagcagtgggagcgcgcgtgcgcgcggccgtgcagcctgggcagtgggtcctgcctgtgacgcgcggcggcggtcggtcctgcctgtaacggcggcggcggctgctgctccagacacctgcggcggcggcggcgaccccgcggcgggcgcggagatgtggcccctggtagcggcgctgttgctgggctcggcgtgctgcggatcagctcagctactatttaataaaacaaaatctgtagaattcacgttttgtaatgacactgtcgtcattccatgctttgttactaatatggaggcacaaaacactactgaagtatacgtaaagtggaaatttaaaggaagagatatttacacctttgatggagctctaaacaagtccactgtccccactgactttagtagtgcaaaaattgaagtctcacaattactaaaaggagatgcctctttgaagatggataagagtgatgctgtctcacacacaggaaactacacttgtgaagtaacagaattaaccagagaaggtgaaacgatcatcgagctaaaatatcgtgttgtttcatggttttctccaaatgaaaatattcttattgttattttcccaatttttgctatactcctgttctggggacagtttggtattaaaacacttaaatatagatccggtggtatggatgagaaaacaattgctttacttgttgctggactagtgatcactgtcattgtcattgttggagccattcttttcgtcccaggtgaatattcattaaagaatgctactggccttggtttaattgtgacttctacagggatattaatattacttcactactatgtgtttagtacagcgattggattaacctccttcgtcattgccatattggttattcaggtgatagcctatatcctcgctgtggttggactgagtctctgtattgcggcgtgtataccaatgcatggccctcttctgatttcaggtttgagtatcttagctctagcacaattacttggactagtttatatgaaatttgtggcttccaatcagaagactatacaacctcctaggaataactgaagtgaagtgatggactccgatttggagagtagtaagacgtgaaaggaatacacttgtgtttaagcaccatggccttgatgattcactgttggggagaagaaacaagaaaagtaactggttgtcacctatgagacccttacgtgattgttagttaagtttttattcaaagcagctgtaatttagttaataaaataattatgatctatgttgtttgcccaattgagatccagttttttgttgttatttttaatcaattaggggcaatagtagaatggacaatttccaagaatgatgcctttcaggtcctagggcctctggcctctaggtaaccagtttaaattggttcagggtgataactacttagcactgccctggtgattacccagagatatctatgaaaaccagtggcttccatcaaacctttgccaactcaggttcacagcagctttgggcagttatggcagtatggcattagctgagaggtgtctgccacttctgggtcaatggaataataaattaagtacaggcaggaatttggttgggagcatcttgtatgatctccgtatgatgtgatattgatggagatagtggtcctcattcttgggggttgccattcccacattcccccttcaacaaacagtgtaacaggtccttcccagatttagggtacttttattgatggatatgttttccttttattcacataaccccttgaaaccctgtcttgtcctcctgttacttgcttctgctgtacaagatgtagcaccttttctcctctttgaacatggtctagtgacacggtagcaccagttgcaggaaggagccagacttgttctcagagcactgtgttcacacttttcagcaaaaatagctatggttgtaacatatgtattcccttcctctgatttgaaggcaaaaatctacagtgtttcttcacttcttttctgatctggggcatgaaaaaagcaagattgaaatttgaactatgagtctcctgcatggcaacaaaatgtgtgtcaccatcaggccaacaggccagcccttgaatggggatttattactgttgtatctatgttgcatgataaacattcatcaccttcctcctgtagtcctgcctcgtactccccttcccctatgattgaaaagtaaacaaaacccacatttcctatcctggttagaagaaaattaatgttctgacagttgtgatcgcctggagtacttttagacttttagcattcgttttttacctgtttgtggatgtgtgtttgtatgtgcatacgtatgagataggcacatgcatcttctgtatggacaaaggtggggtacctacaggagagcaaaggttaattttgtgcttttagtaaaaacatttaaatacaaagttctttattgggtggaattatatttgatgcaaatatttgatcacttaaaacttttaaaacttctaggtaatttgccacgctttttgactgctcaccaataccctgtaaaaatacgtaattcttcctgtttgtgtaataagatattcatatttgtagttgcattaataatagttatttcttagtccatcagatgttcccgtgtgcctcttttatgccaaattgattgtcatatttcatgttgggaccaagtagtttgcccatggcaaacctaaatttatgacctgctgaggcctctcagaaaactgagcatactagcaagacagctcttcttgaaaaaaaaaatatgtatacacaaatatatacgtatatctatatatacgtatgtatatacacacatgtatattcttccttgattgtgtagctgtccaaaataataacatatatagagggagctgtattcctttatacaaatctgatggctcctgcagcactttttccttctgaaaatatttacattttgctaacctagtttgttactttaaaaatcagttttgatgaaaggagggaaaagcagatggacttgaaaaagatccaagctcctattagaaaaggtatgaaaatctttatagtaaaattttttataaactaaagttgtaccttttaatatgtagtaaactctcatttatttggggttcgctcttggatctcatccatccattgtgttctctttaatgctgcctgccttttgaggcattcactgccctagacaatgccaccagagatagtgggggaaatgccagatgaaaccaactcttgctctcactagttgtcagcttctctggataagtgaccacagaagcaggagtcctcctgcttgggcatcattgggccagttccttctctttaaatcagatttgtaatggctcccaaattccatcacatcacatttaaattgcagacagtgttttgcacatcatgtatctgttttgtcccataatatgctttttactccctgatcccagtttctgctgttgactcttccattcagttttatttattgtgtgttctcacagtgacaccatttgtccttttctgcaacaacctttccagctacttttgccaaattctatttgtcttctccttcaaaacattctcctttgcagttcctcttcatctgtgtagctgctcttttgtctcttaacttaccattcctatagtactttatgcatctctgcttagttctattagttttttggccttgctcttctccttgattttaaaattccttctatagctagagcttttctttctttcattctctcttcctgcagtgttttgcatacatcagaagctaggtacataagttaaatgattgagagttggctgtatttagatttatcactttttaatagggtgagcttgagagttttctttctttctgttttttttttttgttttttttttttttttttttttttttttttttgactaatttcacatgctctaaaaaccttcaaaggtgattatttttctcctggaaactccaggtccattctgtttaaatccctaagaatgtcagaattaaaataacagggctatcccgtaattggaaatatttcttttttcaggatgctatagtcaatttagtaagtgaccaccaaattgttatttgcactaacaaagctcaaaacacgataagtttactcctccatctcagtaataaaaattaagctgtaatcaaccttctaggtttctcttgtcttaaaatgggtattcaaaaatggggatctgtggtgtatgtatggaaacacatactccttaatttacctgttgttggaaactggagaaatgattgtcgggcaaccgtttattttttattgtattttatttggttgagggatttttttataaacagttttacttgtgtcatattttaaaattactaactgccatcacctgctggggtcctttgttaggtcattttcagtgactaatagggataatccaggtaactttgaagagatgagcagtgagtgaccaggcagtttttctgcctttagctttgacagttcttaattaagatcattgaagaccagctttctcataaatttctctttttgaaaaaaagaaagcatttgtactaagctcctctgtaagacaacatcttaaatcttaaaagtgttgttatcatgactggtgagagaagaaaacattttgtttttattaaatggagcattatttacaaaaagccattgttgagaattagatcccacatcgtataaatatctattaaccattctaaataaagagaactccagtgttgctatgtgcaagatcctctcttggagcttttttgcatagcaattaaaggtgtgctatttgtcagtagccatttttttgcagtgatttgaagaccaaagttgttttacagctgtgttaccgttaaaggtttttttttttatatgtattaaatcaatttatcactgtttaaagctttgaatatctgcaatctttgccaaggtacttttttatttaaaaaaaaacataactttgtaaatattaccctgtaatattatatatacttaataaaacattttaagctattttgttgggctatttctattgctgctacagcagaccacaagcacatttctgaaaaatttaatttattaatgtatttttaagttgcttatattctaggtaacaatgtaaagaatgatttaaaatattaattatgaattttttgagtataatacccaataagcttttaattagagcagagttttaattaaaagttttaaatcagtc

SEQ ID NO: 12 - protein, 305 aa, Homo sapiens
MWPLVAALLLGSACCGSAQLLFNKTKSVEFTFCNDTVVIPCFVTNMEAQNTTEVYVKWKFKGRDIYTFDGALNKSTVPTDFSSAKIEVSQLLKGDASLKMDKSDAVSHTGNYTCEVTELTREGETIIELKYRVVSWFSPNENILIVIFPIFAILLFWGQFGIKTLKYRSGGMDEKTIALLVAGLVITVIVIVGAILFVPGEYSLKNATGLGLIVTSTGILILLHYYVFSTAIGLTSFVIAILVIQVIAYILAVVGLSLCIAACIPMHGPLLISGLSILALAQLLGLVYMKFVASNQKTIQPPRNN

SEQ ID NO: 13 - DNA, 5078 bp, Homo sapiens
agtgggagcgcgcgtgcgcgcggccgtgcagcctgggcagtgggtcctgcctgtgacgcgcggcggcggtcggtcctgcctgtaacggcggcggcggctgctgctccggacacctgcggcggcggcggcgaccccgcggcgggcgcggagatgtggcccctggtagcggcgctgttgctgggctcggcgtgctgcggatcagctcagctactatttaataaaacaaaatctgtagaattcacgttttgtaatgacactgtcgtcattccatgctttgttactaatatggaggcacaaaacactactgaagtatacgtaaagtggaaatttaaaggaagagatatttacacctttgatggagctctaaacaagtccactgtccccactgactttagtagtgcaaaaattgaagtctcacaattactaaaaggagatgcctctttgaagatggataagagtgatgctgtctcacacacaggaaactacacttgtgaagtaacagaattaaccagagaaggtgaaacgatcatcgagctaaaatatcgtgttgtttcatggttttctccaaatgaaaatattcttattgttattttcccaatttttgctatactcctgttctggggacagtttggtattaaaacacttaaatatagatccggtggtatggatgagaaaacaattgctttacttgttgctggactagtgatcactgtcattgtcattgttggagccattcttttcgtcccaggtgaatattcattaaagaatgctactggccttggtttaattgtgacttctacagggatattaatattacttcactactatgtgtttagtacagcgattggattaacctccttcgtcattgccatattggttattcaggtgatagcctatatcctcgctgtggttggactgagtctctgtattgcggcgtgtataccaatgcatggccctcttctgatttcaggtttgagtatcttagctctagcacaattacttggactagtttatatgaaatttgtggcttccaatcagaagactatacaacctcctaggaaagctgtagaggaaccccttaatgaataactgaagtgaagtgatggactccgatttggagagtagtaagacgtgaaaggaatacacttgtgtttaagcaccatggccttgatgattcactgttggggagaagaaacaagaaaagtaactggttgtcacctatgagacccttacgtgattgttagttaagtttttattcaaagcagctgtaatttagttaataaaataattatgatctatgttgtttgcccaattgagatccagttttttgttgttatttttaatcaattaggggcaatagtagaatggacaatttccaagaatgatgcctttcaggtcctagggcctctggcctctaggtaaccagtttaaattggttcagggtgataactacttagcactgccctggtgattacccagagatatctatgaaaaccagtggcttccatcaaacctttgccaactcaggttcacagcagctttgggcagttatggcagtatggcattagctgagaggtgtctgccacttctgggtcaatggaataataaattaagtacaggcaggaatttggttgggagcatcttgtatgatctccgtatgatgtgatattgatggagatagtggtcctcattcttgggggttgccattcccacattcccccttcaacaaacagtgtaacaggtccttcccagatttagggtacttttattgatggatatgttttccttttattcacataaccccttgaaaccctgtcttgtcctcctgttacttgcttctgctgtacaagatgtagcaccttttctcctctttgaacatggtctagtgacacggtagcaccagttgcaggaaggagccagacttgttctcagagcactgtgttcacacttttcagcaaaaatagctatggttgtaacatatgtattcccttcctctgatttgaaggcaaaaatctacagtgtttcttcacttcttttctgatctggggcatgaaaaaagcaagattgaaatttgaactatgagtctcctgcatggcaacaaaatgtgtgtcaccatcaggccaacaggccagcccttgaatggggatttattactgttgtatctatgttgcatgataaacattcatcaccttcctcctgtagtcctgcctcgtactccccttcccctatgattgaaaagtaaacaaaacccacatttcctatcctggttagaagaaaattaatgttctgacagttgtgatcgcctggagtacttttagacttttagcattcgttttttacctgtttgtggatgtgtgtttgtatgtgcatacgtatgagataggcacatgcatcttctgtatggacaaaggtggggtacctacaggagagcaaaggttaattttgtgcttttagtaaaaacatttaaatacaaagttctttattgggtggaattatatttgatgcaaatatttgatcacttaaaacttttaaaacttctaggtaatttgccacgctttttgactgctcaccaataccctgtaaaaatacgtaattcttcctgtttgtgtaataagatattcatatttgtagttgcattaataatagttatttcttagtccatcagatgttcccgtgtgcctcttttatgccaaattgattgtcatatttcatgttgggaccaagtagtttgcccatggcaaacctaaatttatgacctgctgaggcctctcagaaaactgagcatactagcaagacagctcttcttgaaaaaaaaaatatgtatacacaaatatatacgtatatctatatatacgtatgtatatacacacatgtatattcttccttgattgtgtagctgtccaaaataataacatatatagagggagctgtattcctttatacaaatctgatggctcctgcagcactttttccttctgaaaatatttacattttgctaacctagtttgttactttaaaaatcagttttgatgaaaggagggaaaagcagatggacttgaaaaagatccaagctcctattagaaaaggtatgaaaatctttatagtaaaattttttataaactaaagttgtaccttttaatatgtagtaaactctcatttatttggggttcgctcttggatctcatccatccattgtgttctctttaatgctgcctgccttttgaggcattcactgccctagacaatgccaccagagatagtgggggaaatgccagatgaaaccaactcttgctctcactagttgtcagcttctctggataagtgaccacagaagcaggagtcctcctgcttgggcatcattgggccagttccttctctttaaatcagatttgtaatggctcccaaattccatcacatcacatttaaattgcagacagtgttttgcacatcatgtatctgttttgtcccataatatgctttttactccctgatcccagtttctgctgttgactcttccattcagttttatttattgtgtgttctcacagtgacaccatttgtccttttctgcaacaacctttccagctacttttgccaaattctatttgtcttctccttcaaaacattctcctttgcagttcctcttcatctgtgtagctgctcttttgtctcttaacttaccattcctatagtactttatgcatctctgcttagttctattagttttttggccttgctcttctccttgattttaaaattccttctatagctagagcttttctttctttcattctctcttcctgcagtgttttgcatacatcagaagctaggtacataagttaaatgattgagagttggctgtatttagatttatcactttttaatagggtgagcttgagagttttctttctttctgttttttttttttgttttttttttttttttttttttttttttttttgactaatttcacatgctctaaaaaccttcaaaggtgattatttttctcctggaaactccaggtccattctgtttaaatccctaagaatgtcagaattaaaataacagggctatcccgtaattggaaatatttcttttttcaggatgctatagtcaatttagtaagtgaccaccaaattgttatttgcactaacaaagctcaaaacacgataagtttactcctccatctcagtaataaaaattaagctgtaatcaaccttctaggtttctcttgtcttaaaatgggtattcaaaaatggggatctgtggtgtatgtatggaaacacatactccttaatttacctgttgttggaaactggagaaatgattgtcgggcaaccgtttattttttattgtattttatttggttgagggatttttttataaacagttttacttgtgtcatattttaaaattactaactgccatcacctgctggggtcctttgttaggtcattttcagtgactaatagggataatccaggtaactttgaagagatgagcagtgagtgaccaggcagtttttctgcctttagctttgacagttcttaattaagatcattgaagaccagctttctcataaatttctctttttgaaaaaaagaaagcatttgtactaagctcctctgtaagacaacatcttaaatcttaaaagtgttgttatcatgactggtgagagaagaaaacattttgtttttattaaatggagcattatttacaaaaagccattgttgagaattagatcccacatcgtataaatatctattaaccattctaaataaagagaactccagtgttgctatgtgcaagatcctctcttggagcttttttgcatagcaattaaaggtgtgctatttgtcagtagccatttttttgcagtgatttgaagaccaaagttgttttacagctgtgttaccgttaaaggtttttttttttatatgtattaaatcaatttatcactgtttaaagctttgaatatctgcaatctttgccaaggtacttttttatttaaaaaaaaacataactttgtaaatattaccctgtaatattatatatacttaataaaacattttaagcta

SEQ ID NO: 14 - protein, 312 aa, Homo sapiens
MWPLVAALLLGSACCGSAQLLFNKTKSVEFTFCNDTVVIPCFVTNMEAQNTTEVYVKWKFKGRDIYTFDGALNKSTVPTDFSSAKIEVSQLLKGDASLKMDKSDAVSHTGNYTCEVTELTREGETIIELKYRVVSWFSPNENILIVIFPIFAILLFWGQFGIKTLKYRSGGMDEKTIALLVAGLVITVIVIVGAILFVPGEYSLKNATGLGLIVTSTGILILLHYYVFSTAIGLTSFVIAILVIQVIAYILAVVGLSLCIAACIPMHGPLLISGLSILALAQLLGLVYMKFVASNQKTIQPPRKAVEEPLNE

SEQ ID NO: 15 - DNA, 5346 bp, Homo sapiens
ggggagcaggcgggggagcgggcgggaagcagtgggagcgcgcgtgcgcgcggccgtgcagcctgggcagtgggtcctgcctgtgacgcgcggcggcggtcggtcctgcctgtaacggcggcggcggctgctgctccagacacctgcggcggcggcggcgaccccgcggcgggcgcggagatgtggcccctggtagcggcgctgttgctgggctcggcgtgctgcggatcagctcagctactatttaataaaacaaaatctgtagaattcacgttttgtaatgacactgtcgtcattccatgctttgttactaatatggaggcacaaaacactactgaagtatacgtaaagtggaaatttaaaggaagagatatttacacctttgatggagctctaaacaagtccactgtccccactgactttagtagtgcaaaaattgaagtctcacaattactaaaaggagatgcctctttgaagatggataagagtgatgctgtctcacacacaggaaactacacttgtgaagtaacagaattaaccagagaaggtgaaacgatcatcgagctaaaatatcgtgttgtttcatggttttctccaaatgaaaatattcttattgttattttcccaatttttgctatactcctgttctggggacagtttggtattaaaacacttaaatatagatccggtggtatggatgagaaaacaattgctttacttgttgctggactagtgatcactgtcattgtcattgttggagccattcttttcgtcccaggtgaatattcattaaagaatgctactggccttggtttaattgtgacttctacagggatattaatattacttcactactatgtgtttagtacagcgattggattaacctccttcgtcattgccatattggttattcaggtgatagcctatatcctcgctgtggttggactgagtctctgtattgcggcgtgtataccaatgcatggccctcttctgatttcaggtttgagtatcttagctctagcacaattacttggactagtttatatgaaatttgtggcttccaatcagaagactatacaacctcctaggaaagctgtagaggaaccccttaatgcattcaaagaatcaaaaggaatgatgaatgatgaataactgaagtgaagtgatggactccgatttggagagtagtaagacgtgaaaggaatacacttgtgtttaagcaccatggccttgatgattcactgttggggagaagaaacaagaaaagtaactggttgtcacctatgagacccttacgtgattgttagttaagtttttattcaaagcagctgtaatttagttaataaaataattatgatctatgttgtttgcccaattgagatccagttttttgttgttatttttaatcaattaggggcaatagtagaatggacaatttccaagaatgatgcctttcaggtcctagggcctctggcctctaggtaaccagtttaaattggttcagggtgataactacttagcactgccctggtgattacccagagatatctatgaaaaccagtggcttccatcaaacctttgccaactcaggttcacagcagctttgggcagttatggcagtatggcattagctgagaggtgtctgccacttctgggtcaatggaataataaattaagtacaggcaggaatttggttgggagcatcttgtatgatctccgtatgatgtgatattgatggagatagtggtcctcattcttgggggttgccattcccacattcccccttcaacaaacagtgtaacaggtccttcccagatttagggtacttttattgatggatatgttttccttttattcacataaccccttgaaaccctgtcttgtcctcctgttacttgcttctgctgtacaagatgtagcaccttttctcctctttgaacatggtctagtgacacggtagcaccagttgcaggaaggagccagacttgttctcagagcactgtgttcacacttttcagcaaaaatagctatggttgtaacatatgtattcccttcctctgatttgaaggcaaaaatctacagtgtttcttcacttcttttctgatctggggcatgaaaaaagcaagattgaaatttgaactatgagtctcctgcatggcaacaaaatgtgtgtcaccatcaggccaacaggccagcccttgaatggggatttattactgttgtatctatgttgcatgataaacattcatcaccttcctcctgtagtcctgcctcgtactccccttcccctatgattgaaaagtaaacaaaacccacatttcctatcctggttagaagaaaattaatgttctgacagttgtgatcgcctggagtacttttagacttttagcattcgttttttacctgtttgtggatgtgtgtttgtatgtgcatacgtatgagataggcacatgcatcttctgtatggacaaaggtggggtacctacaggagagcaaaggttaattttgtgcttttagtaaaaacatttaaatacaaagttctttattgggtggaattatatttgatgcaaatatttgatcacttaaaacttttaaaacttctaggtaatttgccacgctttttgactgctcaccaataccctgtaaaaatacgtaattcttcctgtttgtgtaataagatattcatatttgtagttgcattaataatagttatttcttagtccatcagatgttcccgtgtgcctcttttatgccaaattgattgtcatatttcatgttgggaccaagtagtttgcccatggcaaacctaaatttatgacctgctgaggcctctcagaaaactgagcatactagcaagacagctcttcttgaaaaaaaaaatatgtatacacaaatatatacgtatatctatatatacgtatgtatatacacacatgtatattcttccttgattgtgtagctgtccaaaataataacatatatagagggagctgtattcctttatacaaatctgatggctcctgcagcactttttccttctgaaaatatttacattttgctaacctagtttgttactttaaaaatcagttttgatgaaaggagggaaaagcagatggacttgaaaaagatccaagctcctattagaaaaggtatgaaaatctttatagtaaaattttttataaactaaagttgtaccttttaatatgtagtaaactctcatttatttggggttcgctcttggatctcatccatccattgtgttctctttaatgctgcctgccttttgaggcattcactgccctagacaatgccaccagagatagtgggggaaatgccagatgaaaccaactcttgctctcactagttgtcagcttctctggataagtgaccacagaagcaggagtcctcctgcttgggcatcattgggccagttccttctctttaaatcagatttgtaatggctcccaaattccatcacatcacatttaaattgcagacagtgttttgcacatcatgtatctgttttgtcccataatatgctttttactccctgatcccagtttctgctgttgactcttccattcagttttatttattgtgtgttctcacagtgacaccatttgtccttttctgcaacaacctttccagctacttttgccaaattctatttgtcttctccttcaaaacattctcctttgcagttcctcttcatctgtgtagctgctcttttgtctcttaacttaccattcctatagtactttatgcatctctgcttagttctattagttttttggccttgctcttctccttgattttaaaattccttctatagctagagcttttctttctttcattctctcttcctgcagtgttttgcatacatcagaagctaggtacataagttaaatgattgagagttggctgtatttagatttatcactttttaatagggtgagcttgagagttttctttctttctgttttttttttttgttttttttttttttttttttttttttttttttgactaatttcacatgctctaaaaaccttcaaaggtgattatttttctcctggaaactccaggtccattctgtttaaatccctaagaatgtcagaattaaaataacagggctatcccgtaattggaaatatttcttttttcaggatgctatagtcaatttagtaagtgaccaccaaattgttatttgcactaacaaagctcaaaacacgataagtttactcctccatctcagtaataaaaattaagctgtaatcaaccttctaggtttctcttgtcttaaaatgggtattcaaaaatggggatctgtggtgtatgtatggaaacacatactccttaatttacctgttgttggaaactggagaaatgattgtcgggcaaccgtttattttttattgtattttatttggttgagggatttttttataaacagttttacttgtgtcatattttaaaattactaactgccatcacctgctggggtcctttgttaggtcattttcagtgactaatagggataatccaggtaactttgaagagatgagcagtgagtgaccaggcagtttttctgcctttagctttgacagttcttaattaagatcattgaagaccagctttctcataaatttctctttttgaaaaaaagaaagcatttgtactaagctcctctgtaagacaacatcttaaatcttaaaagtgttgttatcatgactggtgagagaagaaaacattttgtttttattaaatggagcattatttacaaaaagccattgttgagaattagatcccacatcgtataaatatctattaaccattctaaataaagagaactccagtgttgctatgtgcaagatcctctcttggagcttttttgcatagcaattaaaggtgtgctatttgtcagtagccatttttttgcagtgatttgaagaccaaagttgttttacagctgtgttaccgttaaaggtttttttttttatatgtattaaatcaatttatcactgtttaaagctttgaatatctgcaatctttgccaaggtacttttttatttaaaaaaaaacataactttgtaaatattaccctgtaatattatatatacttaataaaacattttaagctattttgttgggctatttctattgctgctacagcagaccacaagcacatttctgaaaaatttaatttattaatgtatttttaagttgcttatattctaggtaacaatgtaaagaatgatttaaaatattaattatgaattttttgagtataatacccaataagcttttaattagagcagagttttaattaaaagttttaaatcagtc

SEQ ID NO: 16 - protein, 323 aa, Homo sapiens
MWPLVAALLLGSACCGSAQLLFNKTKSVEFTFCNDTVVIPCFVTNMEAQNTTEVYVKWKFKGRDIYTFDGALNKSTVPTDFSSAKIEVSQLLKGDASLKMDKSDAVSHTGNYTCEVTELTREGETIIELKYRVVSWFSPNENILIVIFPIFAILLFWGQFGIKTLKYRSGGMDEKTIALLVAGLVITVIVIVGAILFVPGEYSLKNATGLGLIVTSTGILILLHYYVFSTAIGLTSFVIAILVIQVIAYILAVVGLSLCIAACIPMHGPLLISGLSILALAQLLGLVYMKFVASNQKTIQPPRKAVEEPLNAFKESKGMMNDE

SEQ ID NO: 17 - protein, 293 aa, Artificial Sequence
  source: /note="Description of Artificial Sequence: Synthetic polypeptide"
MWPLAAALLLGSCCCGSAQLLFNKTKSVEFTFCNDTVVIPCFVTNMEAQNTTEVYVKWKFKGRDIYTFDGALNKSTVPTDFSSAKIEVSQLLKGDASLKMDKSDAVSHTGNYTCEVTELTREGETIIELKYRVVSWFSPNENILIVIFPIFAILLFWGQFGIKTLKYRSGGMDEKTIALLVAGLVITVIVIVGAILFVPGEYSLKNATGLGLIVTSTGILILLHYYVFSTAIGLTSFVIAILVIQVIAYILAVVGLSLCIAACIPMHGPLLISGLSILALAQLLGLVYMKFVE

SEQ ID NO: 18 - protein, 305 aa, Artificial Sequence
  source: /note="Description of Artificial Sequence: Synthetic polypeptide"
MWPLAAALLLGSCCCGSAQLLFNKTKSVEFTFCNDTVVIPCFVTNMEAQNTTEVYVKWKFKGRDIYTFDGALNKSTVPTDFSSAKIEVSQLLKGDASLKMDKSDAVSHTGNYTCEVTELTREGETIIELKYRVVSWFSPNENILIVIFPIFAILLFWGQFGIKTLKYRSGGMDEKTIALLVAGLVITVIVIVGAILFVPGEYSLKNATGLGLIVTSTGILILLHYYVFSTAIGLTSFVIAILVIQVIAYILAVVGLSLCIAACIPMHGPLLISGLSILALAQLLGLVYMKFVASNQRTIQPPRNR

SEQ ID NO: 19 - protein, 312 aa, Artificial Sequence
  source: /note="Description of Artificial Sequence: Synthetic polypeptide"
MWPLAAALLLGSCCCGSAQLLFNKTKSVEFTFCNDTVVIPCFVTNMEAQNTTEVYVKWKFKGRDIYTFDGALNKSTVPTDFSSAKIEVSQLLKGDASLKMDKSDAVSHTGNYTCEVTELTREGETIIELKYRVVSWFSPNENILIVIFPIFAILLFWGQFGIKTLKYRSGGMDEKTIALLVAGLVITVIVIVGAILFVPGEYSLKNATGLGLIVTSTGILILLHYYVFSTAIGLTSFVIAILVIQVIAYILAVVGLSLCIAACIPMHGPLLISGLSILALAQLLGLVYMKFVASNQRTIQPPRKAVEEPLNE

SEQ ID NO: 20 - protein, 323 aa, Artificial Sequence
  source: /note="Description of Artificial Sequence: Synthetic polypeptide"
MWPLAAALLLGSCCCGSAQLLFNKTKSVEFTFCNDTVVIPCFVTNMEAQNTTEVYVKWKFKGRDIYTFDGALNKSTVPTDFSSAKIEVSQLLKGDASLKMDKSDAVSHTGNYTCEVTELTREGETIIELKYRVVSWFSPNENILIVIFPIFAILLFWGQFGIKTLKYRSGGMDEKTIALLVAGLVITVIVIVGAILFVPGEYSLKNATGLGLIVTSTGILILLHYYVFSTAIGLTSFVIAILVIQVIAYILAVVGLSLCIAACIPMHGPLLISGLSILALAQLLGLVYMKFVASNQRTIQPPRKAVEEPLNAFKESKGMMNDE

SEQ ID NO: 21 - DNA, 22 bp, Artificial Sequence
  source: /note="Description of Artificial Sequence: Synthetic primer"
tgcagaagtcactaggaggaat

SEQ ID NO: 22 - DNA, 27 bp, Artificial Sequence
  source: /note="Description of Artificial Sequence: Synthetic probe"
tcagtcaacttcttctgggttgtttcc

SEQ ID NO: 23 - DNA, 23 bp, Artificial Sequence
  source: /note="Description of Artificial Sequence: Synthetic primer"
gtgccagactcactttctatcca

SEQ ID NO: 24 - DNA, 22 bp, Artificial Sequence
  source: /note="Description of Artificial Sequence: Synthetic primer"
tgctgccaatatacggcttctg

SEQ ID NO: 25 - DNA, 26 bp, Artificial Sequence
  source: /note="Description of Artificial Sequence: Synthetic probe"
cagctctcatagccaactatggtgcc

SEQ ID NO: 26 - DNA, 22 bp, Artificial Sequence
  source: /note="Description of Artificial Sequence: Synthetic primer"
tcaagcagagcctggttatctg

SEQ ID NO: 27 - DNA, 23 bp, Artificial Sequence
  source: /note="Description of Artificial Sequence: Synthetic primer"
gtcgtcattccatgctttgttac

SEQ ID NO: 28 - DNA, 30 bp, Artificial Sequence
  source: /note="Description of Artificial Sequence: Synthetic probe"
tggaggcacaaaacactactgaagtatacg

SEQ ID NO: 29 - DNA, 22 bp, Artificial Sequence
  source: /note="Description of Artificial Sequence: Synthetic primer"
ggacagtggacttgtttagagc

SEQ ID NO: 30 - DNA, 21 bp, Artificial Sequence
  source: /note="Description of Artificial Sequence: Synthetic primer"
ggcttggtggctgattgttct

SEQ ID NO: 31 - DNA, 28 bp, Artificial Sequence
  source: /note="Description of Artificial Sequence: Synthetic probe"
agcacccaaactgatatgcctgtatttg

SEQ ID NO: 32 - DNA, 23 bp, Artificial Sequence
  source: /note="Description of Artificial Sequence: Synthetic primer"
tgggaactggtgtttcaagtcta

SEQ ID NO: 33 - DNA, 158 bp, Artificial Sequence
  source: /note="Description of Artificial Sequence: Synthetic polynucleotide"
gcagacatgattacttcagagctttcaaagctagatactgtaccttgcatattccaacacgcgatcgcattttaagattttccatcctagtggaaagatatgatttgattcatcctatttactttgtatattaaagtacagtagaacctgccactttt

SEQ ID NO: 34 - DNA, 160 bp, Artificial Sequence
  source: /note="Description of Artificial Sequence: Synthetic polynucleotide"
ggatccattttaagtaatagaataggatttttaattgttccagtgtttctgtgatagagctgtcctgcacagacctgtttctcgagataacttcgtataatgtatgctatacgaagttatatgcatggcctccgcgccgggttttggcgcctcccgcggg

SEQ ID NO: 35 - DNA, 160 bp, Artificial Sequence
  source: /note="Description of Artificial Sequence: Synthetic polynucleotide"
catgtctggaataacttcgtataatgtatgctatacgaagttatgctagtaactataacggtcctaaggtagcgactagcattagtatggaaggtccgtccactgtccaggttcctcttgcggagctctttgtctctctggactctgtatacactgcttg

SEQ ID NO: 36 - DNA, 239 bp, Artificial Sequence
  source: /note="Description of Artificial Sequence: Synthetic polynucleotide"
ggatccattttaagtaatagaataggatttttaattgttccagtgtttctgtgatagagctgtcctgcacagacctgtttctcgagataacttcgtataatgtatgctatacgaagttatgctagtaactataacggtcctaaggtagcgactagcattagtatggaaggtccgtccactgtccaggttcctcttgcggagctctttgtctctctggactctgtatacactgcttgcat